European Patent Application EP 4 282 426 A1, published November 29, 2023. Title: 一种预防癌症复发的方法和药物组合. Applicant: 厦门特宝生物工程股份有限公司 厦门伯赛基因转录技术有限公司. The sequence listing filed with the application follows.

SEQUENCE LISTING (6 sequences)

SEQ ID NO: 1 - protein, 164 aa, Artificial Sequence
  ARTIFICIAL SEQUENCE
CDLPQTHSLGSRRTLMLLAQMRKISLFSCLKDRHDFGFPQEEFGNQFQKAETIPVLHEMIQQIFNLFSTKDSSAAWDETLLDKFYTELYQQLNDLEACVIQGVGVTEPLMKEDSILAVRKYFQRITLYLKEKKYSPCAWEVVRAEIMRSFSLSTNLQESLRSKE

SEQ ID NO: 2 - protein, 165 aa, ARTIFICIAL SEQUENCE [sequence omitted]

SEQ ID NO: 3 - protein, 167 aa, ARTIFICIAL SEQUENCE
  ARTIFICIAL SEQUENCE
MCDLPQTHSLGNRRALILLAQMRRISPFSCLKDRHDFGFPQEEFDGNQFQKAQAISVLHEMIQQTFNLFSTKDSSAAWDESLLEKFYTELYQQLNDLEACVIQEVGVEETPLMNVDSILAVKKYFQRITLYLTEKKYSPCAWEVVRAEIMRSFSLSTNLQERLRRKE

SEQ ID NO: 4 - protein, 171 aa, Artificial Sequence
  ARTIFICIAL SEQUENCE
GSGGGCDLPQTHSLGNRRALILLAQMRRISPFSCLKDRHDFGFPQEEFDGNQFQKAQAISVLHEMIQQTFNLFSTKDSSAAWDESLLEKFYTELYQQLNDLEACVIQEVGVEETPLMNVDSILAVRKYFQRITLYLTEKKYSPCAWEVVRAEIMRSFSLSTNLQERLRRKD

SEQ ID NO: 5 - protein, 182 aa, ARTIFICIAL SEQUENCE
  ARTIFICIAL SEQUENCE
MGPVPTSKPTTTGKGCHIGRFKSLSPQELASFKKARDALEESLKLKNWSCSSPVFPGNWDLRLLQVRERPVALEAELALTLKVLEAAAGPALEDVLDQPLHTLHHILSQLQACIQPQPTAGPRPRGRLHHWLHRLQEAPKKESAGCLEASVTFNLFRLLTRDLKYVADGNLCLRTSTHPEST

SEQ ID NO: 6 - protein, 162 aa, ARTIFICIAL SEQUENCE
  ARTIFICIAL SEQUENCE
CDLPHTYNLGNKRALTVLEEMRRLPPLSCLKDRKDFGFPLEKVDNQQIQKAQAILVLRDLTQQILNLFTSKDLSATWNATLLDSFCNDLHQQLNDLKACVMQEPPLTQEDSLLAVRTYFHRITVYLRKKKHSLCAWEVIRAEVWRALSSSTNLLARLSEEKE